European Patent Application EP 4 772 532 A1, published July 8, 2026. Title: Lipoproteins containing light-sensitive substances, photodynamic therapy formulations, drug delivery methods, and posterior segment neovascular occlusion methods. Applicant: KYOTO UNIVERSITY. The sequence listing filed with the application follows.

SEQUENCE LISTING (17 sequences)

SEQ ID NO: 1 - protein, 17 aa, Drosophila
RQIKIWFQNRRMKWKKK

SEQ ID NO: 2 - protein, 10 aa, synthetic construct
  REGION 1..10: note = Artificial Sequence
ACDCRGDCFC

SEQ ID NO: 3 - protein, 13 aa, synthetic construct
  REGION 1..13: note = Artificial Sequence
CPKVCPRECESNC

SEQ ID NO: 4 - protein, 7 aa, synthetic construct
  REGION 1..7: note = Artificial Sequence
CNGRCGG

SEQ ID NO: 5 - DNA, 80 bp, synthetic construct
  misc_feature 1..80: note = Artificial Sequence
  source 1..80: mol_type = other DNA
gatgtgagtgtgtgacgagctacgacgtctggtgtaatttataaagacactgtgtatatcaacaacagaacaaggaaagg

SEQ ID NO: 6 - DNA, 24 bp, synthetic construct
  source 1..24: mol_type = other DNA
aagcttagtaccaaagaggctctg

SEQ ID NO: 7 - DNA, 24 bp, synthetic construct
  source 1..24: mol_type = other DNA
ggctagaaacaatagtgaaaacaa

SEQ ID NO: 8 - DNA, 25 bp, synthetic construct
  source 1..25: mol_type = other DNA
agtgacctctggtccttaaacaagg

SEQ ID NO: 9 - DNA, 25 bp, synthetic construct
  source 1..25: mol_type = other DNA
gaggtagagagcaaggatgacttgc

SEQ ID NO: 10 - DNA, 22 bp, synthetic construct
  source 1..22: mol_type = other DNA
tcctcctccatttacagtgaca

SEQ ID NO: 11 - DNA, 24 bp, synthetic construct
  source 1..24: mol_type = other DNA
ttattctcctaaacactgcagctc

SEQ ID NO: 12 - DNA, 24 bp, synthetic construct
  source 1..24: mol_type = other DNA
tgaatctgaagtgatggagaatgg

SEQ ID NO: 13 - DNA, 20 bp, synthetic construct
  source 1..20: mol_type = other DNA
cctatcggagcctagaaccg

SEQ ID NO: 14 - DNA, 21 bp, synthetic construct
  source 1..21: mol_type = other DNA
cccagtacgactgtgacaatg

SEQ ID NO: 15 - DNA, 24 bp, synthetic construct
  source 1..24: mol_type = other DNA
cacagtcttcaaggagatcagcta

SEQ ID NO: 16 - DNA, 20 bp, synthetic construct
  source 1..20: mol_type = other DNA
acggatttggtcgtattggg

SEQ ID NO: 17 - DNA, 20 bp, synthetic construct
  source 1..20: mol_type = other DNA
acggatttggtcgtattggg